European Patent Specification EP 2 970 361 B1, published February 15, 2023. Title: COMPOSITIONS AND METHODS FOR MULTIPLEX NUCLEIC ACIDS SYNTHESIS. Applicant: Gen 9, Inc. Jacobson, Joseph Schindler, Daniel Saaem, Ishtiaq Lawton, Scott Goldberg, Martin  J. Hudson, Micahel E. Kung, Li-yun  A. Application Not yet assigned. The sequence listing filed with the application follows.

SEQUENCE LISTING (8 sequences)

SEQ ID NO: 1 - DNA, 96 bp, Artificial Sequence
  Synthetic construct
tacgcccagtttggtaaggtgtggtagcaaggaaaaaaatgacgctcgtgggttcctacaggagcagaagcacttaagccatgtcgtttttgttac

SEQ ID NO: 2 - DNA, 96 bp, Artificial Sequence
  Synthetic construct
acatggcttaagtgcttctgctcctgtaagaacccacgagcgtcatttttttccttgctaccacaccttaccaaactgggcgtatacgcgtacgcg

SEQ ID NO: 3 - DNA, 96 bp, Artificial Sequence
  Synthetic construct
cccgctttagctacattcggcactagaaaaggacgaaaatgacgctcgtgggttcctacaaatcattgtctgcttaaggaggttttgtaagagttc

SEQ ID NO: 4 - DNA, 96 bp, Artificial Sequence
  Synthetic construct
aacctccttaagcagacaatgatttgtaggaacccacgagcgtcattttcgtccttttctagtgccgaatgtagctaaagcgggtacgcgtacgcg

SEQ ID NO: 5 - DNA, 100 bp, Artificial Sequence
  Synthetic construct
ggcgggtgtaattcgttctcttatgtgactctgtttctcttagcagaaggtagtcgcagtcactccttgaaagctcgcgactactctctctgcgccttct

SEQ ID NO: 6 - DNA, 100 bp, Artificial Sequence
  Synthetic construct
gagagtagtcgcgagctttcaaggagtgactgcgactaccttctgctaagagaaacagagtcacataagagaacgaattacacccgccgtaacaaaaacg

SEQ ID NO: 7 - DNA, 100 bp, Artificial Sequence
  Synthetic construct
ctgctcaaagctgccgaaactcgagtctagcgcaactcggccgttataactgactggtttagcgatttttgcaattcgagctactaaaataaggtttctc

SEQ ID NO: 8 - DNA, 100 bp, Artificial Sequence
  Synthetic construct
tttagtagctcgaattgcaaaaatcgctaaaccagtcagttataacggccgagttgcgctagactcgagtttcggcagctttgagcaggaactcttacaa